European Patent Application EP 4 541 898 A2, published April 23, 2025. Title: Liver-Specific Inducible Promoters and Methods of Use Thereof. Applicant: AskBio Inc. Application EP. The sequence listing filed with the application follows.

SEQUENCE LISTING (91 sequences)

SEQ ID NO: 1 - DNA, 51 bp, Mus musculus
  source 1..51: mol_type = unassigned DNA
tctgtactttcctgaccttggcacagtgccaccatcaacttgcctgacacc

SEQ ID NO: 2 - DNA, 51 bp, Homo sapiens
  source 1..51: mol_type = unassigned DNA
actgtactttcctgaccctgaagaggtggcagcatggactttcctgaacca

SEQ ID NO: 3 - DNA, 16 bp, Mus musculus
  source 1..16: mol_type = unassigned DNA
tgtactttcctgacct

SEQ ID NO: 4 - DNA, 16 bp, Homo sapiens
  source 1..16: mol_type = unassigned DNA
tgtactttcctgaccc

SEQ ID NO: 5 - DNA, 84 bp, synthetic construct
  misc_feature 1..84: note = 3x NR1 sequence (mouse)
  source 1..84: mol_type = other DNA
gatctctgtactttcctgaccttggatcgatctctgtactttcctgaccttggatcgatctctgtactttcctgaccttggatc

SEQ ID NO: 6 - DNA, 84 bp, synthetic construct
  misc_feature 1..84: note = 3x NR1 sequence (human)
  source 1..84: mol_type = other DNA
gatcactgtactttcctgaccctggatcgatcactgtactttcctgaccctggatcgatcactgtactttcctgaccctggatc

SEQ ID NO: 7 - DNA, 262 bp, synthetic construct
  misc_feature 1..262: note = PB1-MinTK
  source 1..262: mol_type = other DNA
tctgtactttcctgaccttggcacagtgccaccatcaacttgcctgacaccgatccggccccgcccagcgtcttgtcattggcgaattcgaacacgcagatgcagtcggggcggcgcggtccgaggtccacttcgcatattaaggtgacgcgtgtggcctcgaacaccgagcgaccctgcagcgacccgcttaacagcgtcaacagcgtgccgcagatctcgaggagcttggcgagattttcaggagctaaggaagctaaac

SEQ ID NO: 8 - DNA, 180 bp, synthetic construct
  misc_feature 1..180: note = PB1-CMV-MP
  source 1..180: mol_type = other DNA
tctgtactttcctgaccttggcacagtgccaccatcaacttgcctgacaccgctgggagttcgtagacggagcgattaatccatatgcaggtctatataagcagagctcgtttagtgaaccgtcagatcgcctagatacgccatccacgctgttttgacctccatagaagatcgccaccc

SEQ ID NO: 9 - DNA, 330 bp, synthetic construct
  misc_feature 1..330: note = PB1-SV40-MP
  source 1..330: mol_type = other DNA
tctgtactttcctgaccttggcacagtgccaccatcaacttgcctgacaccgctgggagttcgtagacggactagcccgggctcgagatctgcgatctgcatctcaattagtcagcaaccatagtcccgcccctaactccgcccatcccgcccctaactccgcccagttccgcccattctccgccccatcgctgactaattttttttatttatgcagaggccgaggccgcctcggcctctgagctattccagaagtagtgaggaggcttttttggaggcctaggcttttgcaaaaagcttggcattccggtactgttggtaaagccaccc

SEQ ID NO: 10 - DNA, 353 bp, synthetic construct
  misc_feature 1..353: note = PB1-1-MinTk (2xPBREM)
  source 1..353: mol_type = other DNA
tctgtactttcctgaccttggcacagtgccaccatcaacttgcctgacacccattactcgcatccattctctctgtactttcctgaccttggcacagtgccaccatcaacttgcctgacaccgctgggagttcgtagacggagatccggccccgcccagcgtcttgtcattggcgaattcgaacacgcagatgcagtcggggcggcgcggtccgaggtccacttcgcatattaaggtgacgcgtgtggcctcgaacaccgagcgaccctgcagcgacccgcttaacagcgtcaacagcgtgccgcagatctcgaggagcttggcgagattttcaggagctaaggaagctaaac

SEQ ID NO: 11 - DNA, 424 bp, synthetic construct
  misc_feature 1..424: note = PB1-2-MinTk (3xPBREM)
  source 1..424: mol_type = other DNA
tctgtactttcctgaccttggcacagtgccaccatcaacttgcctgacacccattactcgcatccattctctctgtactttcctgaccttggcacagtgccaccatcaacttgcctgacaccgcactgaaggtcctcaatcgtctgtactttcctgaccttggcacagtgccaccatcaacttgcctgacaccgctgggagttcgtagacggagatccggccccgcccagcgtcttgtcattggcgaattcgaacacgcagatgcagtcggggcggcgcggtccgaggtccacttcgcatattaaggtgacgcgtgtggcctcgaacaccgagcgaccctgcagcgacccgcttaacagcgtcaacagcgtgccgcagatctcgaggagcttggcgagattttcaggagctaaggaagctaaac

SEQ ID NO: 12 - DNA, 495 bp, synthetic construct
  misc_feature 1..495: note = PB1-3-MinTk
  source 1..495: mol_type = other DNA
tctgtactttcctgaccttggcacagtgccaccatcaacttgcctgacacccattactcgcatccattctctctgtactttcctgaccttggcacagtgccaccatcaacttgcctgacaccgcactgaaggtcctcaatcgtctgtactttcctgaccttggcacagtgccaccatcaacttgcctgacaccctgacctcctgccagcaatatctgtactttcctgaccttggcacagtgccaccatcaacttgcctgacaccgctgggagttcgtagacggagatccggccccgcccagcgtcttgtcattggcgaattcgaacacgcagatgcagtcggggcggcgcggtccgaggtccacttcgcatattaaggtgacgcgtgtggcctcgaacaccgagcgaccctgcagcgacccgcttaacagcgtcaacagcgtgccgcagatctcgaggagcttggcgagattttcaggagctaaggaagctaaac

SEQ ID NO: 13 - DNA, 401 bp, synthetic construct
  misc_feature 1..401: note = PB1-1-SV40
  source 1..401: mol_type = other DNA
tctgtactttcctgaccttggcacagtgccaccatcaacttgcctgacacccattactcgcatccattctctctgtactttcctgaccttggcacagtgccaccatcaacttgcctgacaccgctgggagttcgtagacggactagcccgggctcgagatctgcgatctgcatctcaattagtcagcaaccatagtcccgcccctaactccgcccatcccgcccctaactccgcccagttccgcccattctccgccccatcgctgactaattttttttatttatgcagaggccgaggccgcctcggcctctgagctattccagaagtagtgaggaggcttttttggaggcctaggcttttgcaaaaagcttggcattccggtactgttggtaaagccaccc

SEQ ID NO: 14 - DNA, 472 bp, synthetic construct
  misc_feature 1..472: note = PB1-2-SV40
  source 1..472: mol_type = other DNA
tctgtactttcctgaccttggcacagtgccaccatcaacttgcctgacacccattactcgcatccattctctctgtactttcctgaccttggcacagtgccaccatcaacttgcctgacaccgcactgaaggtcctcaatcgtctgtactttcctgaccttggcacagtgccaccatcaacttgcctgacaccgctgggagttcgtagacggactagcccgggctcgagatctgcgatctgcatctcaattagtcagcaaccatagtcccgcccctaactccgcccatcccgcccctaactccgcccagttccgcccattctccgccccatcgctgactaattttttttatttatgcagaggccgaggccgcctcggcctctgagctattccagaagtagtgaggaggcttttttggaggcctaggcttttgcaaaaagcttggcattccggtactgttggtaaagccaccc

SEQ ID NO: 15 - DNA, 543 bp, synthetic construct
  misc_feature 1..543: note = PB1-3-SV40
  source 1..543: mol_type = other DNA
tctgtactttcctgaccttggcacagtgccaccatcaacttgcctgacacccattactcgcatccattctctctgtactttcctgaccttggcacagtgccaccatcaacttgcctgacaccgcactgaaggtcctcaatcgtctgtactttcctgaccttggcacagtgccaccatcaacttgcctgacaccctgacctcctgccagcaatatctgtactttcctgaccttggcacagtgccaccatcaacttgcctgacaccgctgggagttcgtagacggactagcccgggctcgagatctgcgatctgcatctcaattagtcagcaaccatagtcccgcccctaactccgcccatcccgcccctaactccgcccagttccgcccattctccgccccatcgctgactaattttttttatttatgcagaggccgaggccgcctcggcctctgagctattccagaagtagtgaggaggcttttttggaggcctaggcttttgcaaaaagcttggcattccggtactgttggtaaagccaccc

SEQ ID NO: 16 - DNA, 251 bp, synthetic construct
  misc_feature 1..251: note = PB1-1-CMV
  source 1..251: mol_type = other DNA
tctgtactttcctgaccttggcacagtgccaccatcaacttgcctgacacccattactcgcatccattctctctgtactttcctgaccttggcacagtgccaccatcaacttgcctgacaccgctgggagttcgtagacggagcgattaatccatatgcaggtctatataagcagagctcgtttagtgaaccgtcagatcgcctagatacgccatccacgctgttttgacctccatagaagatcgccaccc

SEQ ID NO: 17 - DNA, 322 bp, synthetic construct
  misc_feature 1..322: note = PB1-2-CMV
  source 1..322: mol_type = other DNA
tctgtactttcctgaccttggcacagtgccaccatcaacttgcctgacacccattactcgcatccattctctctgtactttcctgaccttggcacagtgccaccatcaacttgcctgacaccgcactgaaggtcctcaatcgtctgtactttcctgaccttggcacagtgccaccatcaacttgcctgacaccgctgggagttcgtagacggagcgattaatccatatgcaggtctatataagcagagctcgtttagtgaaccgtcagatcgcctagatacgccatccacgctgttttgacctccatagaagatcgccaccc

SEQ ID NO: 18 - DNA, 393 bp, synthetic construct
  misc_feature 1..393: note = PB1-3-CMV
  source 1..393: mol_type = other DNA
tctgtactttcctgaccttggcacagtgccaccatcaacttgcctgacacccattactcgcatccattctctctgtactttcctgaccttggcacagtgccaccatcaacttgcctgacaccgcactgaaggtcctcaatcgtctgtactttcctgaccttggcacagtgccaccatcaacttgcctgacaccctgacctcctgccagcaatatctgtactttcctgaccttggcacagtgccaccatcaacttgcctgacaccgctgggagttcgtagacggagcgattaatccatatgcaggtctatataagcagagctcgtttagtgaaccgtcagatcgcctagatacgccatccacgctgttttgacctccatagaagatcgccaccc

SEQ ID NO: 19 - DNA, 1023 bp, synthetic construct
  misc_feature 1..1023: note = PB1-MinTK and EPO
  source 1..1023: mol_type = other DNA
ggcctaactggccggtactctgtactttcctgaccttggcacagtgccaccatcaacttgcctgacaccgatccggccccgcccagcgtcttgtcattggcgaattcgaacacgcagatgcagtcggggcggcgcggtccgaggtccacttcgcatattaaggtgacgcgtgtggcctcgaacaccgagcgaccctgcagcgacccgcttaacagcgtcaacagcgtgccgcagatctcgaggagcttggcgagattttcaggagctaaggaagctaaacatgggggtgcacgaatgtcctgcctggctgtggcttctcctgtccctgctgtcgctccctctgggcctcccagtcctgggcgccccaccacgcctcatctgtgacagccgagtcctggagaggtacctcttggaggccaaggaggccgagaatatcacgacgggctgtgctgaacactgcagcttgaatgagaatatcactgtcccagacaccaaagttaatttctatgcctggaagaggatggaggtcgggcagcaggccgtagaagtctggcagggcctggccctgctgtcggaagctgtcctgcggggccaggccctgttggtcaactcttcccagccgtgggagcccctgcagctgcatgtggataaagccgtcagtggccttcgcagcctcaccactctgcttcgggctctgggagcccagaaggaagccatctcccctccagatgcggcctcagctgctccactccgaacaatcactgctgacactttccgcaaactcttccgagtctactccaatttcctccggggaaagctgaagctgtacacaggggaggcctgcaggacaggggacagatgatctagagtcggggcggccggccgcttcgagcagacatgataagatacattgatgagtttggacaaaccacaactagaatgcagtgaaaaaaatgctttatttgtgaaatttgtgatgctattgctttatttgtaaccattataagctgcaataaacaagtt

SEQ ID NO: 20 - DNA, 16 bp, synthetic construct
  misc_feature 1..16: note = NR1 motif from PBREM
  misc_feature 16: note = n is a, c, g, or t
  source 1..16: mol_type = other DNA
tgtactttcctgaccn

SEQ ID NO: 21 - DNA, 17 bp, synthetic construct
  misc_feature 1..17: note = sequence preferably comprised in a functional variant of a PBREM element
  misc_feature 17: note = n is a, c, g, or t
  source 1..17: mol_type = other DNA
ctgtactttcctgaccn

SEQ ID NO: 22 - DNA, 17 bp, synthetic construct
  misc_feature 1..17: note = sequence preferably comprised in a functional variant of a PBREM element
  source 1..17: mol_type = other DNA
ctgtactttcctgaccy

SEQ ID NO: 23 - DNA, 17 bp, synthetic construct
  misc_feature 1..17: note = sequence preferably comprised in a functional variant of a PBREM element
  source 1..17: mol_type = other DNA
ctgtactttcctgacct

SEQ ID NO: 24 - DNA, 17 bp, synthetic construct
  misc_feature 1..17: note = sequence preferably comprised in a functional variant of a PBREM element
  source 1..17: mol_type = other DNA
ctgtactttcctgaccc

SEQ ID NO: 25 - DNA, 20 bp, synthetic construct
  misc_feature 1..20: note = sequence suitably comprised in a functional variant of a PBREM sequence
  misc_feature 1: note = n is a, c, g, or t
  misc_feature 18: note = n is a, c, g, or t
  source 1..20: mol_type = other DNA
nctgtactttcctgaccntg

SEQ ID NO: 26 - DNA, 20 bp, synthetic construct
  misc_feature 1..20: note = sequence suitably comprised in a functional variant of a PBREM sequence
  source 1..20: mol_type = other DNA
wctgtactttcctgaccytg

SEQ ID NO: 27 - DNA, 20 bp, synthetic construct
  misc_feature 1..20: note = sequence suitably comprised in a functional variant of a PBREM sequence
  source 1..20: mol_type = other DNA
tctgtactttcctgaccttg

SEQ ID NO: 28 - DNA, 20 bp, synthetic construct
  misc_feature 1..20: note = sequence suitably comprised in a functional variant of a PBREM sequence
  source 1..20: mol_type = other DNA
actgtactttcctgaccctg

SEQ ID NO: 29 - DNA, 16 bp, synthetic construct
  misc_feature 1..16: note = sequence suitably comprised in a functional variant of a PBREM sequence
  misc_feature 16: note = optional spacer
  misc_feature 16: note = n is a, c, g, or t
  source 1..16: mol_type = other DNA
tgtactttcctgaccn

SEQ ID NO: 30 - DNA, 17 bp, synthetic construct
  misc_feature 1..17: note = sequence suitably comprised in a functional variant of a PBREM sequence
  misc_feature 17: note = optional spacer
  misc_feature 17: note = n is a, c, g, or t
  source 1..17: mol_type = other DNA
ctgtactttcctgaccn

SEQ ID NO: 31 - DNA, 20 bp, synthetic construct
  misc_feature 1..20: note = sequence suitably comprised in a functional variant of a PBREM sequence
  misc_feature 1: note = n is a, c, g, or t
  misc_feature 18: note = n is a, c, g, or t
  misc_feature 20: note = optional spacer
  source 1..20: mol_type = other DNA
nctgtactttcctgaccntg

SEQ ID NO: 32 - DNA, 32 bp, synthetic construct
  misc_feature 1..32: note = sequence suitably comprised in a functional variant of a PBREM sequence
  misc_feature 16..17: note = optional spacer
  misc_feature 16: note = n is a, c, g, or t
  misc_feature 32: note = n is a, c, g, or t
  source 1..32: mol_type = other DNA
tgtactttcctgaccntgtactttcctgaccn

SEQ ID NO: 33 - DNA, 48 bp, synthetic construct
  misc_feature 1..48: note = sequence suitably comprised in a functional variant of a PBREM sequence
  misc_feature 16..17: note = optional spacer
  misc_feature 16: note = n is a, c, g, or t
  misc_feature 32: note = n is a, c, g, or t
  misc_feature 32..33: note = optional spacer
  misc_feature 48: note = n is a, c, g, or t
  source 1..48: mol_type = other DNA
tgtactttcctgaccntgtactttcctgaccntgtactttcctgaccn

SEQ ID NO: 34 - DNA, 34 bp, synthetic construct
  misc_feature 1..34: note = sequence suitably comprised in a functional variant of a PBREM sequence
  misc_feature 17..18: note = optional spacer
  misc_feature 17: note = n is a, c, g, or t
  misc_feature 34: note = n is a, c, g, or t
  source 1..34: mol_type = other DNA
ctgtactttcctgaccnctgtactttcctgaccn

SEQ ID NO: 35 - DNA, 51 bp, synthetic construct
  misc_feature 1..51: note = sequence suitably comprised in a functional variant of a PBREM sequence
  misc_feature 17..18: note = optional spacer
  misc_feature 17: note = n is a, c, g, or t
  misc_feature 34: note = n is a, c, g, or t
  misc_feature 34..35: note = optional spacer
  misc_feature 51: note = n is a, c, g, or t
  source 1..51: mol_type = other DNA
ctgtactttcctgaccnctgtactttcctgaccnctgtactttcctgaccn

SEQ ID NO: 36 - DNA, 40 bp, synthetic construct
  misc_feature 1..40: note = sequence suitably comprised in a functional variant of a PBREM sequence
  misc_feature 1: note = n is a, c, g, or t
  misc_feature 18: note = n is a, c, g, or t
  misc_feature 20..21: note = optional spacer
  misc_feature 21: note = n is a, c, g, or t
  misc_feature 38: note = n is a, c, g, or t
  source 1..40: mol_type = other DNA
nctgtactttcctgaccntgnctgtactttcctgaccntg

SEQ ID NO: 37 - DNA, 60 bp, synthetic construct
  misc_feature 1..60: note = sequence suitably comprised in a functional variant of a PBREM sequence
  misc_feature 1: note = n is a, c, g, or t
  misc_feature 18: note = n is a, c, g, or t
  misc_feature 20..21: note = optional spacer
  misc_feature 21: note = n is a, c, g, or t
  misc_feature 38: note = n is a, c, g, or t
  misc_feature 40..41: note = optional spacer
  misc_feature 41: note = n is a, c, g, or t
  misc_feature 58: note = n is a, c, g, or t
  source 1..60: mol_type = other DNA
nctgtactttcctgaccntgnctgtactttcctgaccntgnctgtactttcctgaccntg

SEQ ID NO: 38 - DNA, 60 bp, synthetic construct
  misc_feature 1..60: note = sequence suitably comprised in a functional variant of a PBREM sequence
  misc_feature 20..21: note = optional spacer
  misc_feature 40..41: note = optional spacer
  source 1..60: mol_type = other DNA
tctgtactttcctgaccttgtctgtactttcctgaccttgtctgtactttcctgaccttg

SEQ ID NO: 39 - DNA, 60 bp, synthetic construct
  misc_feature 1..60: note = sequence suitably comprised in a functional variant of a PBREM sequence
  misc_feature 20..21: note = optional spacer
  misc_feature 40..41: note = optional spacer
  source 1..60: mol_type = other DNA
actgtactttcctgaccctgactgtactttcctgaccctgactgtactttcctgaccctg

SEQ ID NO: 40 - skipped

SEQ ID NO: 41 - DNA, 51 bp, synthetic construct
  misc_feature 1..51: note = sequence preferably comprised in a functional variant of a PBREM sequence
  misc_feature 1: note = n is a, c, g, or t
  misc_feature 18: note = n is a, c, g, or t
  misc_feature 21..25: note = n is a, c, g, or t
  misc_feature 29: note = n is a, c, g, or t
  misc_feature 32: note = n is a, c, g, or t
  misc_feature 36..37: note = n is a, c, g, or t
  misc_feature 42: note = n is a, c, g, or t
  misc_feature 48..49: note = n is a, c, g, or t
  misc_feature 51: note = n is a, c, g, or t
  source 1..51: mol_type = other DNA
nctgtactttcctgaccntgnnnnngtgncancatnnacttncctganncn

SEQ ID NO: 42 - DNA, 102 bp, synthetic construct
  misc_feature 1..102: note = CRM
  misc_feature 1: note = n is a, c, g, or t
  misc_feature 18: note = n is a, c, g, or t
  misc_feature 21..25: note = n is a, c, g, or t
  misc_feature 29: note = n is a, c, g, or t
  misc_feature 32: note = n is a, c, g, or t
  misc_feature 36..37: note = n is a, c, g, or t
  misc_feature 42: note = n is a, c, g, or t
  misc_feature 48..49: note = n is a, c, g, or t
  misc_feature 51..52: note = optional spacer
  misc_feature 51: note = n is a, c, g, or t
  misc_feature 52: note = n is a, c, g, or t
  misc_feature 69: note = n is a, c, g, or t
  misc_feature 72..76: note = n is a, c, g, or t
  misc_feature 80: note = n is a, c, g, or t
  misc_feature 83: note = n is a, c, g, or t
  misc_feature 87..88: note = n is a, c, g, or t
  misc_feature 93: note = n is a, c, g, or t
  misc_feature 99..100: note = n is a, c, g, or t
  misc_feature 102: note = n is a, c, g, or t
  source 1..102: mol_type = other DNA
nctgtactttcctgaccntgnnnnngtgncancatnnacttncctganncnnctgtactttcctgaccntgnnnnngtgncancatnnacttncctganncn

SEQ ID NO: 43 - DNA, 153 bp, synthetic construct
  misc_feature 1..153: note = CRM
  misc_feature 1: note = n is a, c, g, or t
  misc_feature 18: note = n is a, c, g, or t
  misc_feature 21..25: note = n is a, c, g, or t
  misc_feature 29: note = n is a, c, g, or t
  misc_feature 32: note = n is a, c, g, or t
  misc_feature 36..37: note = n is a, c, g, or t
  misc_feature 42: note = n is a, c, g, or t
  misc_feature 48..49: note = n is a, c, g, or t
  misc_feature 51..52: note = optional spacer
  misc_feature 51: note = n is a, c, g, or t
  misc_feature 52: note = n is a, c, g, or t
  misc_feature 69: note = n is a, c, g, or t
  misc_feature 72..76: note = n is a, c, g, or t
  misc_feature 80: note = n is a, c, g, or t
  misc_feature 83: note = n is a, c, g, or t
  misc_feature 87..88: note = n is a, c, g, or t
  misc_feature 93: note = n is a, c, g, or t
  misc_feature 99..100: note = n is a, c, g, or t
  misc_feature 102: note = n is a, c, g, or t
  misc_feature 102..103: note = optional spacer
  misc_feature 103: note = n is a, c, g, or t
  misc_feature 120: note = n is a, c, g, or t
  misc_feature 123..127: note = n is a, c, g, or t
  misc_feature 131: note = n is a, c, g, or t
  misc_feature 134: note = n is a, c, g, or t
  misc_feature 138..139: note = n is a, c, g, or t
  misc_feature 144: note = n is a, c, g, or t
  misc_feature 150..151: note = n is a, c, g, or t
  misc_feature 153: note = n is a, c, g, or t
  source 1..153: mol_type = other DNA
nctgtactttcctgaccntgnnnnngtgncancatnnacttncctganncnnctgtactttcctgaccntgnnnnngtgncancatnnacttncctganncnnctgtactttcctgaccntgnnnnngtgncancatnnacttncctganncn

SEQ ID NO: 44 - DNA, 102 bp, synthetic construct
  misc_feature 1..102: note = CRM
  misc_feature 51..52: note = optional spacer
  source 1..102: mol_type = other DNA
tctgtactttcctgaccttggcacagtgccaccatcaacttgcctgacacctctgtactttcctgaccttggcacagtgccaccatcaacttgcctgacacc

SEQ ID NO: 45 - DNA, 153 bp, synthetic construct
  misc_feature 1..153: note = CRM
  misc_feature 51..52: note = optional spacer
  misc_feature 102..103: note = optional spacer
  source 1..153: mol_type = other DNA
tctgtactttcctgaccttggcacagtgccaccatcaacttgcctgacacctctgtactttcctgaccttggcacagtgccaccatcaacttgcctgacacctctgtactttcctgaccttggcacagtgccaccatcaacttgcctgacacc

SEQ ID NO: 46 - DNA, 153 bp, synthetic construct
  misc_feature 1..153: note = CRM
  misc_feature 51..52: note = optional spacer
  misc_feature 102..103: note = optional spacer
  source 1..153: mol_type = other DNA
actgtactttcctgaccctgaagaggtggcagcatggactttcctgaaccaactgtactttcctgaccctgaagaggtggcagcatggactttcctgaaccaactgtactttcctgaccctgaagaggtggcagcatggactttcctgaacca

SEQ ID NO: 47 - DNA, 102 bp, synthetic construct
  misc_feature 1..102: note = CRM
  misc_feature 51..52: note = optional spacer
  source 1..102: mol_type = other DNA
actgtactttcctgaccctgaagaggtggcagcatggactttcctgaaccaactgtactttcctgaccctgaagaggtggcagcatggactttcctgaacca

SEQ ID NO: 48 - DNA, 5716 bp, synthetic construct
  misc_feature 1..5716: note = pAAV-ZsGreen original plasmid
  source 1..5716: mol_type = other DNA
agcgcccaatacgcaaaccgcctctccccgcgcgttggccgattcattaatgcagctggcacgacaggtttcccgactggaaagcgggcagtgagcgcaacgcaattaatgtgagttagctcactcattaggcaccccaggctttacactttatgcttccggctcgtatgttgtgtggaattgtgagcggataacaatttcacacaggaaacagctatgaccatgattacgaattgcctgcaggcagctgcgcgctcgctcgctcactgaggccgcccgggcaaagcccgggcgtcgggcgacctttggtcgcccggcctcagtgagcgagcgagcgcgcagagagggagtggccaactccatcactaggggttcctatcgatatcaagctttaatagtaatcaattacggggtcattagttcatagcccatatatggagttccgcgttacataacttacggtaaatggcccgcctggctgaccgcccaacgacccccgcccattgacgtcaataatgacgtatgttcccatagtaacgccaatagggactttccattgacgtcaatgggtggagtatttacggtaaactgcccacttggcagtacatcaagtgtatcatatgccaagtacgccccctattgacgtcaatgacggtaaatggcccgcctggcattatgcccagtacatgaccttatgggactttcctacttggcagtacatctacgtattagtcatcgctattaccatggtgatgcggttttggcagtacatcaatgggcgtggatagcggtttgactcacggggatttccaagtctccaccccattgacgtcaatgggagtttgttttggcaccaaaatcaacgggactttccaaaatgtcgtaacaactccgccccattgacgcaaatgggcggtaggcgtgtacggtgggaggtctatataagcagagctggtttagtggatatccttaagggcccagccggcccgaatcccggccgggaacggtgcattggaacgcggattccccgtgccaagagtgacgtaagtaccgcctatagagtctataggcccacaaaaaatgctttcttcttttaatatacttttttgtttatcttatttctaatactttccctaatctctttctttcagggcaataatgatacaatgtatcatgcctctttgcaccattctaaagaataacagtgataatttctgggttaaggcaatagcaatatttctgcatataaatatttctgcatataaattgtaactgatgtaagaggtttcatattgctaatagcagctacaatccagctaccattctgcttttattttatggttgggataaggctggattattctgagtccaagctaggcccttttgctaatcatgttcatacctcttatcttcctcccacagctcctgggcaacgtgctggtctgtgtgctggcccatcactttggcaaagaattgggattcgcgagaattcgccaccatggcccagtccaagcacggcctgaccaaggagatgaccatgaagtaccgcatggagggctgcgtggacggccacaagttcgtgatcaccggcgagggcatcggctaccccttcaagggcaagcaggccatcaacctgtgcgtggtggagggcggccccttgcccttcgccgaggacatcttgtccgccgccttcatgtacggcaaccgcgtgttcaccgagtacccccaggacatcgtcgactacttcaagaactcctgccccgccggctacacctgggaccgctccttcctgttcgaggacggcgccgtgtgcatctgcaacgccgacatcaccgtgagcgtggaggagaactgcatgtaccacgagtccaagttctacggcgtgaacttccccgccgacggccccgtgatgaagaagatgaccgacaactgggagccctcctgcgagaagatcatccccgtgcccaagcagggcatcttgaagggcgacgtgagcatgtacctgctgctgaaggacggtggccgcttgcgctgccagttcgacaccgtgtacaaggccaagtccgtgccccgcaagatgcccgactggcacttcatccagcacaagctgacccgcgaggaccgcagcgacgccaagaaccagaagtggcacctgaccgagcacgccatcgcctccggctccgccttgccctgataaggatccacgggtggcatccctgtgacccctccccagtgcctctcctggccctggaagttgccactccagtgcccaccagccttgtcctaataaaattaagttgcatcattttgtctgactaggtgtccttctataatattatggggtggaggggggtggtatggagcaaggggcaagttgggaagacaacctgtagggcctgcggggtctattgggaaccaagctggagtgcagtggcacaatcttggctcactgcaatctccgcctcctgggttcaagcgattctcctgcctcagcctcccgagttgttgggattccaggcatgcatgaccaggctcagctaatttttgtttttttggtagagacggggtttcaccatattggccaggctggtctccaactcctaatctcaggtgatctacccaccttggcctcccaaattgctgggattacaggcgtgaaccactgctcccttccctgtccttatcgatagatctaggaacccctagtgatggagttggccactccctctctgcgcgctcgctcgctcactgaggccgggcgaccaaaggtcgcccgacgcccgggctttgcccgggcggcctcagtgagcgagcgagcgcgcagctgcctgcaggcagcttggcactggccgtcgttttacaacgtcgtgactgggaaaaccctggcgttacccaacttaatcgccttgcagcacatccccctttcgccagctggcgtaatagcgaagaggcccgcaccgatcgcccttcccaacagttgcgcagcctgaatggcgaatggcgcctgatgcggtattttctccttacgcatctgtgcggtatttcacaccgcatacgtcaaagcaaccatagtacgcgccctgtagcggcgcattaagcgcggcgggtgtggtggttacgcgcagcgtgaccgctacacttgccagcgccctagcgcccgctcctttcgctttcttcccttcctttctcgccacgttcgccggctttccccgtcaagctctaaatcgggggctccctttagggttccgatttagtgctttacggcacctcgaccccaaaaaacttgatttgggtgatggttcacgtagtgggccatcgccctgatagacggtttttcgccctttgacgttggagtccacgttctttaatagtggactcttgttccaaactggaacaacactcaaccctatctcgggctattcttttgatttataagggattttgccgatttcggcctattggttaaaaaatgagctgatttaacaaaaatttaacgcgaattttaacaaaatattaacgtttacaattttatggtgcactctcagtacaatctgctctgatgccgcatagttaagccagccccgacacccgccaacacccgctgacgcgccctgacgggcttgtctgctcccggcatccgcttacagacaagctgtgaccgtctccgggagctgcatgtgtcagaggttttcaccgtcatcaccgaaacgcgcgagacgaaagggcctcgtgatacgcctatttttataggttaatgtcatgataataatggtttcttagacgtcaggtggcacttttcggggaaatgtgcgcggaacccctatttgtttatttttctaaatacattcaaatatgtatccgctcatgagacaataaccctgataaatgcttcaataatattgaaaaaggaagagtatgagtattcaacatttccgtgtcgcccttattcccttttttgcggcattttgccttcctgtttttgctcacccagaaacgctggtgaaagtaaaagatgctgaagatcagttgggtgcacgagtgggttacatcgaactggatctcaacagcggtaagatccttgagagttttcgccccgaagaacgttttccaatgatgagcacttttaaagttctgctatgtggcgcggtattatcccgtattgacgccgggcaagagcaactcggtcgccgcatacactattctcagaatgacttggttgagtactcaccagtcacagaaaagcatcttacggatggcatgacagtaagagaattatgcagtgctgccataaccatgagtgataacactgcggccaacttacttctgacaacgatcggaggaccgaaggagctaaccgcttttttgcacaacatgggggatcatgtaactcgccttgatcgttgggaaccggagctgaatgaagccataccaaacgacgagcgtgacaccacgatgcctgtagcaatggcaacaacgttgcgcaaactattaactggcgaactacttactctagcttcccggcaacaattaatagactggatggaggcggataaagttgcaggaccacttctgcgctcggcccttccggctggctggtttattgctgataaatctggagccggtgagcgtgggtctcgcggtatcattgcagcactggggccagatggtaagccctcccgtatcgtagttatctacacgacggggagtcaggcaactatggatgaacgaaatagacagatcgctgagataggtgcctcactgattaagcattggtaactgtcagaccaagtttactcatatatactttagattgatttaaaacttcatttttaatttaaaaggatctaggtgaagatcctttttgataatctcatgaccaaaatcccttaacgtgagttttcgttccactgagcgtcagaccccgtagaaaagatcaaaggatcttcttgagatcctttttttctgcgcgtaatctgctgcttgcaaacaaaaaaaccaccgctaccagcggtggtttgtttgccggatcaagagctaccaactctttttccgaaggtaactggcttcagcagagcgcagataccaaatactgttcttctagtgtagccgtagttaggccaccacttcaagaactctgtagcaccgcctacatacctcgctctgctaatcctgttaccagtggctgctgccagtggcgataagtcgtgtcttaccgggttggactcaagacgatagttaccggataaggcgcagcggtcgggctgaacggggggttcgtgcacacagcccagcttggagcgaacgacctacaccgaactgagatacctacagcgtgagctatgagaaagcgccacgcttcccgaagggagaaaggcggacaggtatccggtaagcggcagggtcggaacaggagagcgcacgagggagcttccagggggaaacgcctggtatctttatagtcctgtcgggtttcgccacctctgacttgagcgtcgatttttgtgatgctcgtcaggggggcggagcctatggaaaaacgccagcaacgcggcctttttacggttcctggccttttgctggccttttgctcacatgttctttcctgcgttatcccctgattctgtggataaccgtattaccgcctttgagtgagctgataccgctcgccgcagccgaacgaccgagcgcagcgagtcagtgagcgaggaagcggaag

SEQ ID NO: 49 - DNA, 5857 bp, synthetic construct
  misc_feature 1..5857: note = pAAV-PB1-MinTk
  source 1..5857: mol_type = other DNA
tgcctgcaggcagctgcgcgctcgctcgctcactgaggccgcccgggcaaagcccgggcgtcgggcgacctttggtcgcccggcctcagtgagcgagcgagcgcgcagagagggagtggccaactccatcactaggggttcctatcgatatcaagcttctgtactttcctgaccttggcacagtgccaccatcaacttgcctgacaccgatccggccccgcccagcgtcttgtcattggcgaattcgaacacgcagatgcagtcggggcggcgcggtccgaggtccacttcgcatattaaggtgacgcgtgtggcctcgaacaccgagcgaccctgcagcgacccgcttaacagcgtcaacagcgtgccgcagatctcgaggagcttggcgagattttcaggagctaaggaagctaaacatggaagatgccaaaaacattaagaagggcccagcgccattctacccactcgaagacgggaccgccggcgagcagctgcacaaagccatgaagcgctacgccctggtgcccggcaccatcgcctttaccgacgcacatatcgaggtggacattacctacgccgagtacttcgagatgagcgttcggctggcagaagctatgaagcgctatgggctgaatacaaaccatcggatcgtggtgtgcagcgagaatagcttgcagttcttcatgcccgtgttgggtgccctgttcatcggtgtggctgtggccccagctaacgacatctacaacgagcgcgagctgctgaacagcatgggcatcagccagcccaccgtcgtattcgtgagcaagaaagggctgcaaaagatcctcaacgtgcaaaagaagctaccgatcatacaaaagatcatcatcatggatagcaagaccgactaccagggcttccaaagcatgtacaccttcgtgacttcccatttgccacccggcttcaacgagtacgacttcgtgcccgagagcttcgaccgggacaaaaccatcgccctgatcatgaacagtagtggcagtaccggattgcccaagggcgtagccctaccgcaccgcaccgcttgtgtccgattcagtcatgcccgcgaccccatcttcggcaaccagatcatccccgacaccgctatcctcagcgtggtgccatttcaccacggcttcggcatgttcaccacgctgggctacttgatctgcggctttcgggtcgtgctcatgtaccgcttcgaggaggagctattcttgcgcagcttgcaagactataagattcaatctgccctgctggtgcccacactatttagcttcttcgctaagagcactctcatcgacaagtacgacctaagcaacttgcacgagatcgccagcggcggggcgccgctcagcaaggaggtaggtgaggccgtggccaaacgcttccacctaccaggcatccgccagggctacggcctgacagaaacaaccagcgccattctgatcacccccgaaggggacgacaagcctggcgcagtaggcaaggtggtgcccttcttcgaggctaaggtggtggacttggacaccggtaagacactgggtgtgaaccagcgcggcgagctgtgcgtccgtggccccatgatcatgagcggctacgttaacaaccccgaggctacaaacgctctcatcgacaaggacggctggctgcacagcggcgacatcgcctactgggacgaggacgagcacttcttcatcgtggaccggctgaagagcctgatcaaatacaagggctaccaggtagccccagccgaactggagagcatcctgctgcaacaccccaacatcttcgacgccggggtcgccggcctgcccgacgacgatgccggcgagctgcccgccgcagtcgtcgtgctggaacacggtaaaaccatgaccgagaaggagatcgtggactatgtggccagccaggttacaaccgccaagaagctgcgcggtggtgttgtgttcgtggacgaggtgcctaaaggactgaccggcaagttggacgcccgcaagatccgcgagattctcattaaggccaagaagggcggcaagatcgccgtgtaatcgcgagaattctctagagtcgacactagtgcggatccacgggtggcatccctgtgacccctccccagtgcctctcctggccctggaagttgccactccagtgcccaccagccttgtcctaataaaattaagttgcatcattttgtctgactaggtgtccttctataatattatggggtggaggggggtggtatggagcaaggggcaagttgggaagacaacctgtagggcctgcggggtctattgggaaccaagctggagtgcagtggcacaatcttggctcactgcaatctccgcctcctgggttcaagcgattctcctgcctcagcctcccgagttgttgggattccaggcatgcatgaccaggctcagctaatttttgtttttttggtagagacggggtttcaccatattggccaggctggtctccaactcctaatctcaggtgatctacccaccttggcctcccaaattgctgggattacaggcgtgaaccactgctcccttccctgtccttatcgatagatctaggaacccctagtgatggagttggccactccctctctgcgcgctcgctcgctcactgaggccgggcgaccaaaggtcgcccgacgcccgggctttgcccgggcggcctcagtgagcgagcgagcgcgcagctgcctgcaggcagcttggcactggccgtcgttttacaacgtcgtgactgggaaaaccctggcgttacccaacttaatcgccttgcagcacatccccctttcgccagctggcgtaatagcgaagaggcccgcaccgatcgcccttcccaacagttgcgcagcctgaatggcgaatggcgcctgatgcggtattttctccttacgcatctgtgcggtatttcacaccgcatacgtcaaagcaaccatagtacgcgccctgtagcggcgcattaagcgcggcgggtgtggtggttacgcgcagcgtgaccgctacacttgccagcgccctagcgcccgctcctttcgctttcttcccttcctttctcgccacgttcgccggctttccccgtcaagctctaaatcgggggctccctttagggttccgatttagtgctttacggcacctcgaccccaaaaaacttgatttgggtgatggttcacgtagtgggccatcgccctgatagacggtttttcgccctttgacgttggagtccacgttctttaatagtggactcttgttccaaactggaacaacactcaaccctatctcgggctattcttttgatttataagggattttgccgatttcggcctattggttaaaaaatgagctgatttaacaaaaatttaacgcgaattttaacaaaatattaacgtttacaattttatggtgcactctcagtacaatctgctctgatgccgcatagttaagccagccccgacacccgccaacacccgctgacgcgccctgacgggcttgtctgctcccggcatccgcttacagacaagctgtgaccgtctccgggagctgcatgtgtcagaggttttcaccgtcatcaccgaaacgcgcgagacgaaagggcctcgtgatacgcctatttttataggttaatgtcatgataataatggtttcttagacgtcaggtggcacttttcggggaaatgtgcgcggaacccctatttgtttatttttctaaatacattcaaatatgtatccgctcatgagacaataaccctgataaatgcttcaataatattgaaaaaggaagagtatgagtattcaacatttccgtgtcgcccttattcccttttttgcggcattttgccttcctgtttttgctcacccagaaacgctggtgaaagtaaaagatgctgaagatcagttgggtgcacgagtgggttacatcgaactggatctcaacagcggtaagatccttgagagttttcgccccgaagaacgttttccaatgatgagcacttttaaagttctgctatgtggcgcggtattatcccgtattgacgccgggcaagagcaactcggtcgccgcatacactattctcagaatgacttggttgagtactcaccagtcacagaaaagcatcttacggatggcatgacagtaagagaattatgcagtgctgccataaccatgagtgataacactgcggccaacttacttctgacaacgatcggaggaccgaaggagctaaccgcttttttgcacaacatgggggatcatgtaactcgccttgatcgttgggaaccggagctgaatgaagccataccaaacgacgagcgtgacaccacgatgcctgtagcaatggcaacaacgttgcgcaaactattaactggcgaactacttactctagcttcccggcaacaattaatagactggatggaggcggataaagttgcaggaccacttctgcgctcggcccttccggctggctggtttattgctgataaatctggagccggtgagcgtgggtctcgcggtatcattgcagcactggggccagatggtaagccctcccgtatcgtagttatctacacgacggggagtcaggcaactatggatgaacgaaatagacagatcgctgagataggtgcctcactgattaagcattggtaactgtcagaccaagtttactcatatatactttagattgatttaaaacttcatttttaatttaaaaggatctaggtgaagatcctttttgataatctcatgaccaaaatcccttaacgtgagttttcgttccactgagcgtcagaccccgtagaaaagatcaaaggatcttcttgagatcctttttttctgcgcgtaatctgctgcttgcaaacaaaaaaaccaccgctaccagcggtggtttgtttgccggatcaagagctaccaactctttttccgaaggtaactggcttcagcagagcgcagataccaaatactgttcttctagtgtagccgtagttaggccaccacttcaagaactctgtagcaccgcctacatacctcgctctgctaatcctgttaccagtggctgctgccagtggcgataagtcgtgtcttaccgggttggactcaagacgatagttaccggataaggcgcagcggtcgggctgaacggggggttcgtgcacacagcccagcttggagcgaacgacctacaccgaactgagatacctacagcgtgagctatgagaaagcgccacgcttcccgaagggagaaaggcggacaggtatccggtaagcggcagggtcggaacaggagagcgcacgagggagcttccagggggaaacgcctggtatctttatagtcctgtcgggtttcgccacctctgacttgagcgtcgatttttgtgatgctcgtcaggggggcggagcctatggaaaaacgccagcaacgcggcctttttacggttcctggccttttgctggccttttgctcacatgttctttcctgcgttatcccctgattctgtggataaccgtattaccgcctttgagtgagctgataccgctcgccgcagccgaacgaccgagcgcagcgagtcagtgagcgaggaagcggaagagcgcccaatacgcaaaccgcctctccccgcgcgttggccgattcattaatgcagctggcacgacaggtttcccgactggaaagcgggcagtgagcgcaacgcaattaatgtgagttagctcactcattaggcaccccaggctttacactttatgcttccggctcgtatgttgtgtggaattgtgagcggataacaatttcacacaggaaacagctatgaccatgattacgaat

SEQ ID NO: 50 - DNA, 6044 bp, synthetic construct
  misc_feature 1..6044: note = pAAV-PB1-2-MinTk
  source 1..6044: mol_type = other DNA
gcctgcaggcagctgcgcgctcgctcgctcactgaggccgcccgggcaaagcccgggcgtcgggcgacctttggtcgcccggcctcagtgagcgagcgagcgcgcagagagggagtggccaactccatcactaggggttcctatcgatatcaagcttttctctggcctaactggccggtactctgtactttcctgaccttggcacagtgccaccatcaacttgcctgacacccattactcgcatccattctctctgtactttcctgaccttggcacagtgccaccatcaacttgcctgacaccgcactgaaggtcctcaatcgtctgtactttcctgaccttggcacagtgccaccatcaacttgcctgacaccgctgggagttcgtagacggagatccggccccgcccagcgtcttgtcattggcgaattcgaacacgcagatgcagtcggggcggcgcggtccgaggtccacttcgcatattaaggtgacgcgtgtggcctcgaacaccgagcgaccctgcagcgacccgcttaacagcgtcaacagcgtgccgcagatctcgaggagcttggcgagattttcaggagctaaggaagctaaacatggaagatgccaaaaacattaagaagggcccagcgccattctacccactcgaagacgggaccgccggcgagcagctgcacaaagccatgaagcgctacgccctggtgcccggcaccatcgcctttaccgacgcacatatcgaggtggacattacctacgccgagtacttcgagatgagcgttcggctggcagaagctatgaagcgctatgggctgaatacaaaccatcggatcgtggtgtgcagcgagaatagcttgcagttcttcatgcccgtgttgggtgccctgttcatcggtgtggctgtggccccagctaacgacatctacaacgagcgcgagctgctgaacagcatgggcatcagccagcccaccgtcgtattcgtgagcaagaaagggctgcaaaagatcctcaacgtgcaaaagaagctaccgatcatacaaaagatcatcatcatggatagcaagaccgactaccagggcttccaaagcatgtacaccttcgtgacttcccatttgccacccggcttcaacgagtacgacttcgtgcccgagagcttcgaccgggacaaaaccatcgccctgatcatgaacagtagtggcagtaccggattgcccaagggcgtagccctaccgcaccgcaccgcttgtgtccgattcagtcatgcccgcgaccccatcttcggcaaccagatcatccccgacaccgctatcctcagcgtggtgccatttcaccacggcttcggcatgttcaccacgctgggctacttgatctgcggctttcgggtcgtgctcatgtaccgcttcgaggaggagctattcttgcgcagcttgcaagactataagattcaatctgccctgctggtgcccacactatttagcttcttcgctaagagcactctcatcgacaagtacgacctaagcaacttgcacgagatcgccagcggcggggcgccgctcagcaaggaggtaggtgaggccgtggccaaacgcttccacctaccaggcatccgccagggctacggcctgacagaaacaaccagcgccattctgatcacccccgaaggggacgacaagcctggcgcagtaggcaaggtggtgcccttcttcgaggctaaggtggtggacttggacaccggtaagacactgggtgtgaaccagcgcggcgagctgtgcgtccgtggccccatgatcatgagcggctacgttaacaaccccgaggctacaaacgctctcatcgacaaggacggctggctgcacagcggcgacatcgcctactgggacgaggacgagcacttcttcatcgtggaccggctgaagagcctgatcaaatacaagggctaccaggtagccccagccgaactggagagcatcctgctgcaacaccccaacatcttcgacgccggggtcgccggcctgcccgacgacgatgccggcgagctgcccgccgcagtcgtcgtgctggaacacggtaaaaccatgaccgagaaggagatcgtggactatgtggccagccaggttacaaccgccaagaagctgcgcggtggtgttgtgttcgtggacgaggtgcctaaaggactgaccggcaagttggacgcccgcaagatccgcgagattctcattaaggccaagaagggcggcaagatcgccgtgtaatcgcgagaattctctagagtcgacactagtgcggatccacgggtggcatccctgtgacccctccccagtgcctctcctggccctggaagttgccactccagtgcccaccagccttgtcctaataaaattaagttgcatcattttgtctgactaggtgtccttctataatattatggggtggaggggggtggtatggagcaaggggcaagttgggaagacaacctgtagggcctgcggggtctattgggaaccaagctggagtgcagtggcacaatcttggctcactgcaatctccgcctcctgggttcaagcgattctcctgcctcagcctcccgagttgttgggattccaggcatgcatgaccaggctcagctaatttttgtttttttggtagagacggggtttcaccatattggccaggctggtctccaactcctaatctcaggtgatctacccaccttggcctcccaaattgctgggattacaggcgtgaaccactgctcccttccctgtccttatcgatagatctaggaacccctagtgatggagttggccactccctctctgcgcgctcgctcgctcactgaggccgggcgaccaaaggtcgcccgacgcccgggctttgcccgggcggcctcagtgagcgagcgagcgcgcagctgcctgcaggcagcttggcactggccgtcgttttacaacgtcgtgactgggaaaaccctggcgttacccaacttaatcgccttgcagcacatccccctttcgccagctggcgtaatagcgaagaggcccgcaccgatcgcccttcccaacagttgcgcagcctgaatggcgaatggcgcctgatgcggtattttctccttacgcatctgtgcggtatttcacaccgcatacgtcaaagcaaccatagtacgcgccctgtagcggcgcattaagcgcggcgggtgtggtggttacgcgcagcgtgaccgctacacttgccagcgccctagcgcccgctcctttcgctttcttcccttcctttctcgccacgttcgccggctttccccgtcaagctctaaatcgggggctccctttagggttccgatttagtgctttacggcacctcgaccccaaaaaacttgatttgggtgatggttcacgtagtgggccatcgccctgatagacggtttttcgccctttgacgttggagtccacgttctttaatagtggactcttgttccaaactggaacaacactcaaccctatctcgggctattcttttgatttataagggattttgccgatttcggcctattggttaaaaaatgagctgatttaacaaaaatttaacgcgaattttaacaaaatattaacgtttacaattttatggtgcactctcagtacaatctgctctgatgccgcatagttaagccagccccgacacccgccaacacccgctgacgcgccctgacgggcttgtctgctcccggcatccgcttacagacaagctgtgaccgtctccgggagctgcatgtgtcagaggttttcaccgtcatcaccgaaacgcgcgagacgaaagggcctcgtgatacgcctatttttataggttaatgtcatgataataatggtttcttagacgtcaggtggcacttttcggggaaatgtgcgcggaacccctatttgtttatttttctaaatacattcaaatatgtatccgctcatgagacaataaccctgataaatgcttcaataatattgaaaaaggaagagtatgagtattcaacatttccgtgtcgcccttattcccttttttgcggcattttgccttcctgtttttgctcacccagaaacgctggtgaaagtaaaagatgctgaagatcagttgggtgcacgagtgggttacatcgaactggatctcaacagcggtaagatccttgagagttttcgccccgaagaacgttttccaatgatgagcacttttaaagttctgctatgtggcgcggtattatcccgtattgacgccgggcaagagcaactcggtcgccgcatacactattctcagaatgacttggttgagtactcaccagtcacagaaaagcatcttacggatggcatgacagtaagagaattatgcagtgctgccataaccatgagtgataacactgcggccaacttacttctgacaacgatcggaggaccgaaggagctaaccgcttttttgcacaacatgggggatcatgtaactcgccttgatcgttgggaaccggagctgaatgaagccataccaaacgacgagcgtgacaccacgatgcctgtagcaatggcaacaacgttgcgcaaactattaactggcgaactacttactctagcttcccggcaacaattaatagactggatggaggcggataaagttgcaggaccacttctgcgctcggcccttccggctggctggtttattgctgataaatctggagccggtgagcgtgggtctcgcggtatcattgcagcactggggccagatggtaagccctcccgtatcgtagttatctacacgacggggagtcaggcaactatggatgaacgaaatagacagatcgctgagataggtgcctcactgattaagcattggtaactgtcagaccaagtttactcatatatactttagattgatttaaaacttcatttttaatttaaaaggatctaggtgaagatcctttttgataatctcatgaccaaaatcccttaacgtgagttttcgttccactgagcgtcagaccccgtagaaaagatcaaaggatcttcttgagatcctttttttctgcgcgtaatctgctgcttgcaaacaaaaaaaccaccgctaccagcggtggtttgtttgccggatcaagagctaccaactctttttccgaaggtaactggcttcagcagagcgcagataccaaatactgttcttctagtgtagccgtagttaggccaccacttcaagaactctgtagcaccgcctacatacctcgctctgctaatcctgttaccagtggctgctgccagtggcgataagtcgtgtcttaccgggttggactcaagacgatagttaccggataaggcgcagcggtcgggctgaacggggggttcgtgcacacagcccagcttggagcgaacgacctacaccgaactgagatacctacagcgtgagctatgagaaagcgccacgcttcccgaagggagaaaggcggacaggtatccggtaagcggcagggtcggaacaggagagcgcacgagggagcttccagggggaaacgcctggtatctttatagtcctgtcgggtttcgccacctctgacttgagcgtcgatttttgtgatgctcgtcaggggggcggagcctatggaaaaacgccagcaacgcggcctttttacggttcctggccttttgctggccttttgctcacatgttctttcctgcgttatcccctgattctgtggataaccgtattaccgcctttgagtgagctgataccgctcgccgcagccgaacgaccgagcgcagcgagtcagtgagcgaggaagcggaagagcgcccaatacgcaaaccgcctctccccgcgcgttggccgattcattaatgcagctggcacgacaggtttcccgactggaaagcgggcagtgagcgcaacgcaattaatgtgagttagctcactcattaggcaccccaggctttacactttatgcttccggctcgtatgttgtgtggaattgtgagcggataacaatttcacacaggaaacagctatgaccatgattacgaatt

SEQ ID NO: 51 - DNA, 4242 bp, synthetic construct
  misc_feature 1..4242: note = pGL4.10 backbone vector
  source 1..4242: mol_type = other DNA
ggcctaactggccggtacctgagctcgctagcctcgaggatatcaagatctggcctcggcggccaagcttggcaatccggtactgttggtaaagccaccatggaagatgccaaaaacattaagaagggcccagcgccattctacccactcgaagacgggaccgccggcgagcagctgcacaaagccatgaagcgctacgccctggtgcccggcaccatcgcctttaccgacgcacatatcgaggtggacattacctacgccgagtacttcgagatgagcgttcggctggcagaagctatgaagcgctatgggctgaatacaaaccatcggatcgtggtgtgcagcgagaatagcttgcagttcttcatgcccgtgttgggtgccctgttcatcggtgtggctgtggccccagctaacgacatctacaacgagcgcgagctgctgaacagcatgggcatcagccagcccaccgtcgtattcgtgagcaagaaagggctgcaaaagatcctcaacgtgcaaaagaagctaccgatcatacaaaagatcatcatcatggatagcaagaccgactaccagggcttccaaagcatgtacaccttcgtgacttcccatttgccacccggcttcaacgagtacgacttcgtgcccgagagcttcgaccgggacaaaaccatcgccctgatcatgaacagtagtggcagtaccggattgcccaagggcgtagccctaccgcaccgcaccgcttgtgtccgattcagtcatgcccgcgaccccatcttcggcaaccagatcatccccgacaccgctatcctcagcgtggtgccatttcaccacggcttcggcatgttcaccacgctgggctacttgatctgcggctttcgggtcgtgctcatgtaccgcttcgaggaggagctattcttgcgcagcttgcaagactataagattcaatctgccctgctggtgcccacactatttagcttcttcgctaagagcactctcatcgacaagtacgacctaagcaacttgcacgagatcgccagcggcggggcgccgctcagcaaggaggtaggtgaggccgtggccaaacgcttccacctaccaggcatccgccagggctacggcctgacagaaacaaccagcgccattctgatcacccccgaaggggacgacaagcctggcgcagtaggcaaggtggtgcccttcttcgaggctaaggtggtggacttggacaccggtaagacactgggtgtgaaccagcgcggcgagctgtgcgtccgtggccccatgatcatgagcggctacgttaacaaccccgaggctacaaacgctctcatcgacaaggacggctggctgcacagcggcgacatcgcctactgggacgaggacgagcacttcttcatcgtggaccggctgaagagcctgatcaaatacaagggctaccaggtagccccagccgaactggagagcatcctgctgcaacaccccaacatcttcgacgccggggtcgccggcctgcccgacgacgatgccggcgagctgcccgccgcagtcgtcgtgctggaacacggtaaaaccatgaccgagaaggagatcgtggactatgtggccagccaggttacaaccgccaagaagctgcgcggtggtgttgtgttcgtggacgaggtgcctaaaggactgaccggcaagttggacgcccgcaagatccgcgagattctcattaaggccaagaagggcggcaagatcgccgtgtaataattctagagtcggggcggccggccgcttcgagcagacatgataagatacattgatgagtttggacaaaccacaactagaatgcagtgaaaaaaatgctttatttgtgaaatttgtgatgctattgctttatttgtaaccattataagctgcaataaacaagttaacaacaacaattgcattcattttatgtttcaggttcagggggaggtgtgggaggttttttaaagcaagtaaaacctctacaaatgtggtaaaatcgataaggatccgtcgaccgatgcccttgagagccttcaacccagtcagctccttccggtgggcgcggggcatgactatcgtcgccgcacttatgactgtcttctttatcatgcaactcgtaggacaggtgccggcagcgctcttccgcttcctcgctcactgactcgctgcgctcggtcgttcggctgcggcgagcggtatcagctcactcaaaggcggtaatacggttatccacagaatcaggggataacgcaggaaagaacatgtgagcaaaaggccagcaaaaggccaggaaccgtaaaaaggccgcgttgctggcgtttttccataggctccgcccccctgacgagcatcacaaaaatcgacgctcaagtcagaggtggcgaaacccgacaggactataaagataccaggcgtttccccctggaagctccctcgtgcgctctcctgttccgaccctgccgcttaccggatacctgtccgcctttctcccttcgggaagcgtggcgctttctcatagctcacgctgtaggtatctcagttcggtgtaggtcgttcgctccaagctgggctgtgtgcacgaaccccccgttcagcccgaccgctgcgccttatccggtaactatcgtcttgagtccaacccggtaagacacgacttatcgccactggcagcagccactggtaacaggattagcagagcgaggtatgtaggcggtgctacagagttcttgaagtggtggcctaactacggctacactagaagaacagtatttggtatctgcgctctgctgaagccagttaccttcggaaaaagagttggtagctcttgatccggcaaacaaaccaccgctggtagcggtggtttttttgtttgcaagcagcagattacgcgcagaaaaaaaggatctcaagaagatcctttgatcttttctacggggtctgacgctcagtggaacgaaaactcacgttaagggattttggtcatgagattatcaaaaaggatcttcacctagatccttttaaattaaaaatgaagttttaaatcaatctaaagtatatatgagtaaacttggtctgacagcggccgcaaatgctaaaccactgcagtggttaccagtgcttgatcagtgaggcaccgatctcagcgatctgcctatttcgttcgtccatagtggcctgactccccgtcgtgtagatcactacgattcgtgagggcttaccatcaggccccagcgcagcaatgatgccgcgagagccgcgttcaccggcccccgatttgtcagcaatgaaccagccagcagggagggccgagcgaagaagtggtcctgctactttgtccgcctccatccagtctatgagctgctgtcgtgatgctagagtaagaagttcgccagtgagtagtttccgaagagttgtggccattgctactggcatcgtggtatcacgctcgtcgttcggtatggcttcgttcaactctggttcccagcggtcaagccgggtcacatgatcacccatattatgaagaaatgcagtcagctccttagggcctccgatcgttgtcagaagtaagttggccgcggtgttgtcgctcatggtaatggcagcactacacaattctcttaccgtcatgccatccgtaagatgcttttccgtgaccggcgagtactcaaccaagtcgttttgtgagtagtgtatacggcgaccaagctgctcttgcccggcgtctatacgggacaacaccgcgccacatagcagtactttgaaagtgctcatcatcgggaatcgttcttcggggcggaaagactcaaggatcttgccgctattgagatccagttcgatatagcccactcttgcacccagttgatcttcagcatcttttactttcaccagcgtttcggggtgtgcaaaaacaggcaagcaaaatgccgcaaagaagggaatgagtgcgacacgaaaatgttggatgctcatactcgtcctttttcaatattattgaagcatttatcagggttactagtacgtctctcaaggataagtaagtaatattaaggtacgggaggtattggacaggccgcaataaaatatctttattttcattacatctgtgtgttggttttttgtgtgaatcgatagtactaacatacgctctccatcaaaacaaaacgaaacaaaacaaactagcaaaataggctgtccccagtgcaagtgcaggtgccagaacatttctct

SEQ ID NO: 52 - DNA, 584 bp, synthetic construct
  misc_feature 1..584: note = CMV-IE comparative promoter
  source 1..584: mol_type = other DNA
gacattgattattgactagttattaatagtaatcaattacggggtcattagttcatagcccatatatggagttccgcgttacataacttacggtaaatggcccgcctggctgaccgcccaacgacccccgcccattgacgtcaataatgacgtatgttcccatagtaacgccaatagggactttccattgacgtcaatgggtggagtatttacggtaaactgcccacttggcagtacatcaagtgtatcatatgccaagtacgccccctattgacgtcaatgacggtaaatggcccgcctggcattatgcccagtacatgaccttatgggactttcctacttggcagtacatctacgtattagtcatcgctattaccatggtgatgcggttttggcagtacatcaatgggcgtggatagcggtttgactcacggggatttccaagtctccaccccattgacgtcaatgggagtttgttttggcaccaaaatcaacgggactttccaaaatgtcgtaacaactccgccccattgacgcaaatgggcggtaggcgtgtacggtgggaggtctatataagcagagct

SEQ ID NO: 53 - DNA, 8191 bp, synthetic construct
  misc_feature 1..8191: note = pcDNA6.0 beta-galactosidase transfection control
  source 1..8191: mol_type = other DNA
gacggatcgggagatctcccgatcccctatggtgcactctcagtacaatctgctctgatgccgcatagttaagccagtatctgctccctgcttgtgtgttggaggtcgctgagtagtgcgcgagcaaaatttaagctacaacaaggcaaggcttgaccgacaattgcatgaagaatctgcttagggttaggcgttttgcgctgcttcgcgatgtacgggccagatatacgcgttgacattgattattgactagttattaatagtaatcaattacggggtcattagttcatagcccatatatggagttccgcgttacataacttacggtaaatggcccgcctggctgaccgcccaacgacccccgcccattgacgtcaataatgacgtatgttcccatagtaacgccaatagggactttccattgacgtcaatgggtggagtatttacggtaaactgcccacttggcagtacatcaagtgtatcatatgccaagtacgccccctattgacgtcaatgacggtaaatggcccgcctggcattatgcccagtacatgaccttatgggactttcctacttggcagtacatctacgtattagtcatcgctattaccatggtgatgcggttttggcagtacatcaatgggcgtggatagcggtttgactcacggggatttccaagtctccaccccattgacgtcaatgggagtttgttttggcaccaaaatcaacgggactttccaaaatgtcgtaacaactccgccccattgacgcaaatgggcggtaggcgtgtacggtgggaggtctatataagcagagctctctggctaactagagaacccactgcttactggcttatcgaaattaatacgactcactatagggagacccaagctggctagcgtttaaacttaagcttggtaccgagctcggatccactagtccagtgtggtggaattctgcagatcgaaacgatgatagatcccgtcgttttacaacgtcgtgactgggaaaaccctggcgttacccaacttaatcgccttgcagcacatccccctttcgccagctggcgtaatagcgaagaggcccgcaccgatcgcccttcccaacagttgcgcagcctgaatggcgaatggcgctttgcctggtttccggcaccagaagcggtgccggaaagctggctggagtgcgatcttcctgaggccgatactgtcgtcgtcccctcaaactggcagatgcacggttacgatgcgcccatctacaccaacgtgacctatcccattacggtcaatccgccgtttgttcccacggagaatccgacgggttgttactcgctcacatttaatgttgatgaaagctggctacaggaaggccagacgcgaattatttttgatggcgttaactcggcgtttcatctgtggtgcaacgggcgctgggtcggttacggccaggacagtcgtttgccgtctgaatttgacctgagcgcatttttacgcgccggagaaaaccgcctcgcggtgatggtgctgcgctggagtgacggcagttatctggaagatcaggatatgtggcggatgagcggcattttccgtgacgtctcgttgctgcataaaccgactacacaaatcagcgatttccatgttgccactcgctttaatgatgatttcagccgcgctgtactggaggctgaagttcagatgtgcggcgagttgcgtgactacctacgggtaacagtttctttatggcagggtgaaacgcaggtcgccagcggcaccgcgcctttcggcggtgaaattatcgatgagcgtggtggttatgccgatcgcgtcacactacgtctgaacgtcgaaaacccgaaactgtggagcgccgaaatcccgaatctctatcgtgcggtggttgaactgcacaccgccgacggcacgctgattgaagcagaagcctgcgatgtcggtttccgcgaggtgcggattgaaaatggtctgctgctgctgaacggcaagccgttgctgattcgaggcgttaaccgtcacgagcatcatcctctgcatggtcaggtcatggatgagcagacgatggtgcaggatatcctgctgatgaagcagaacaactttaacgccgtgcgctgttcgcattatccgaaccatccgctgtggtacacgctgtgcgaccgctacggcctgtatgtggtggatgaagccaatattgaaacccacggcatggtgccaatgaatcgtctgaccgatgatccgcgctggctaccggcgatgagcgaacgcgtaacgcgaatggtgcagcgcgatcgtaatcacccgagtgtgatcatctggtcgctggggaatgaatcaggccacggcgctaatcacgacgcgctgtatcgctggatcaaatctgtcgatccttcccgcccggtgcagtatgaaggcggcggagccgacaccacggccaccgatattatttgcccgatgtacgcgcgcgtggatgaagaccagcccttcccggctgtgccgaaatggtccatcaaaaaatggctttcgctacctggagagacgcgcccgctgatcctttgcgaatacgcccacgcgatgggtaacagtcttggcggtttcgctaaatactggcaggcgtttcgtcagtatccccgtttacagggcggcttcgtctgggactgggtggatcagtcgctgattaaatatgatgaaaacggcaacccgtggtcggcttacggcggtgattttggcgatacgccgaacgatcgccagttctgtatgaacggtctggtctttgccgaccgcacgccgcatccagcgctgacggaagcaaaacaccagcagcagtttttccagttccgtttatccgggcaaaccatcgaagtgaccagcgaatacctgttccgtcatagcgataacgagctcctgcactggatggtggcgctggatggtaagccgctggcaagcggtgaagtgcctctggatgtcgctccacaaggtaaacagttgattgaactgcctgaactaccgcagccggagagcgccgggcaactctggctcacagtacgcgtagtgcaaccgaacgcgaccgcatggtcagaagccgggcacatcagcgcctggcagcagtggcgtctggcggaaaacctcagtgtgacgctccccgccgcgtcccacgccatcccgcatctgaccaccagcgaaatggatttttgcatcgagctgggtaataagcgttggcaatttaaccgccagtcaggctctctttcacagatgtggattggcgataaaaaccaactgctgacgccgctgcgcgatcagttcacccgtgcaccgctggataacgacattggcgtaagtgaagcgacccgcattgaccctaacgcctgggtcgaacgctggaaggcggcgggccattaccaggccgaagcagcgttgttgcagtgcacggcagatacacttgctgatgcggtgctgattacgaccgctcacgcgtggcagcatcaggggaaaaccttatttatcagccggaaaacctaccggattgatggtagtggtcaaatggcgattaccgttgatgttgaagtggcgagcgatacaccgcatccggcgcggattggcctgaactgccagctggcgcaggtagcagagcgggtaaactggctcggattagggccgcaagaaaactatcccgaccgccttactgccgcctgttttgaccgctgggatctgccattgtcagacatgtataccccgtacgtcttcccgagcgaaaacggtctgcgctgcgggacgcgcgaattgaattatggcccacaccagtggcgcggcgacttccagttcaacatcagccgctacagtcaacagcaactgatggaaaccagccatcgccatctgctgcacgcggaagaaggcacatggctgaatatcgacggtttccatatggggattggtggcgacgactcctggagcccgtcagtatcggcggaattccagctgagcgccggtcgctaccattaccagttggtctggtgtcaaaaagcggccgctcgaggtcacccattcgaaggtaagcctatccctaaccctctcctcggtctcgattctacgcgtaccggtcatcatcaccatcaccattgagtttaaacccgctgatcagcctcgactgtgccttctagttgccagccatctgttgtttgcccctcccccgtgccttccttgaccctggaaggtgccactcccactgtcctttcctaataaaatgaggaaattgcatcgcattgtctgagtaggtgtcattctattctggggggtggggtggggcaggacagcaagggggaggattgggaagacaatagcaggcatgctggggatgcggtgggctctatggcttctgaggcggaaagaaccagctggggctctagggggtatccccacgcgccctgtagcggcgcattaagcgcggcgggtgtggtggttacgcgcagcgtgaccgctacacttgccagcgccctagcgcccgctcctttcgctttcttcccttcctttctcgccacgttcgccggctttccccgtcaagctctaaatcgggggctccctttagggttccgatttagtgctttacggcacctcgaccccaaaaaacttgattagggtgatggttcacgtagtgggccatcgccctgatagacggtttttcgccctttgacgttggagtccacgttctttaatagtggactcttgttccaaactggaacaacactcaaccctatctcggtctattcttttgatttataagggattttgccgatttcggcctattggttaaaaaatgagctgatttaacaaaaatttaacgcgaattaattctgtggaatgtgtgtcagttagggtgtggaaagtccccaggctccccagcaggcagaagtatgcaaagcatgcatctcaattagtcagcaaccaggtgtggaaagtccccaggctccccagcaggcagaagtatgcaaagcatgcatctcaattagtcagcaaccatagtcccgcccctaactccgcccatcccgcccctaactccgcccagttccgcccattctccgccccatggctgactaattttttttatttatgcagaggccgaggccgcctctgcctctgagctattccagaagtagtgaggaggcttttttggaggcctaggcttttgcaaaaagctcccgggagcttgtatatccattttcggatctgatcagcacgtgttgacaattaatcatcggcatagtatatcggcatagtataatacgacaaggtgaggaactaaaccatggccaagcctttgtctcaagaagaatccaccctcattgaaagagcaacggctacaatcaacagcatccccatctctgaagactacagcgtcgccagcgcagctctctctagcgacggccgcatcttcactggtgtcaatgtatatcattttactgggggaccttgtgcagaactcgtggtgctgggcactgctgctgctgcggcagctggcaacctgacttgtatcgtcgcgatcggaaatgagaacaggggcatcttgagcccctgcggacggtgccgacaggtgcttctcgatctgcatcctgggatcaaagccatagtgaaggacagtgatggacagccgacggcagttgggattcgtgaattgctgccctctggttatgtgtgggagggctaagcacttcgtggccgaggagcaggactgacacgtgctacgagatttcgattccaccgccgccttctatgaaaggttgggcttcggaatcgttttccgggacgccggctggatgatcctccagcgcggggatctcatgctggagttcttcgcccaccccaacttgtttattgcagcttataatggttacaaataaagcaatagcatcacaaatttcacaaataaagcatttttttcactgcattctagttgtggtttgtccaaactcatcaatgtatcttatcatgtctgtataccgtcgacctctagctagagcttggcgtaatcatggtcatagctgtttcctgtgtgaaattgttatccgctcacaattccacacaacatacgagccggaagcataaagtgtaaagcctggggtgcctaatgagtgagctaactcacattaattgcgttgcgctcactgcccgctttccagtcgggaaacctgtcgtgccagctgcattaatgaatcggccaacgcgcggggagaggcggtttgcgtattgggcgctcttccgcttcctcgctcactgactcgctgcgctcggtcgttcggctgcggcgagcggtatcagctcactcaaaggcggtaatacggttatccacagaatcaggggataacgcaggaaagaacatgtgagcaaaaggccagcaaaaggccaggaaccgtaaaaaggccgcgttgctggcgtttttccataggctccgcccccctgacgagcatcacaaaaatcgacgctcaagtcagaggtggcgaaacccgacaggactataaagataccaggcgtttccccctggaagctccctcgtgcgctctcctgttccgaccctgccgcttaccggatacctgtccgcctttctcccttcgggaagcgtggcgctttctcatagctcacgctgtaggtatctcagttcggtgtaggtcgttcgctccaagctgggctgtgtgcacgaaccccccgttcagcccgaccgctgcgccttatccggtaactatcgtcttgagtccaacccggtaagacacgacttatcgccactggcagcagccactggtaacaggattagcagagcgaggtatgtaggcggtgctacagagttcttgaagtggtggcctaactacggctacactagaagaacagtatttggtatctgcgctctgctgaagccagttaccttcggaaaaagagttggtagctcttgatccggcaaacaaaccaccgctggtagcggtggtttttttgtttgcaagcagcagattacgcgcagaaaaaaaggatctcaagaagatcctttgatcttttctacggggtctgacgctcagtggaacgaaaactcacgttaagggattttggtcatgagattatcaaaaaggatcttcacctagatccttttaaattaaaaatgaagttttaaatcaatctaaagtatatatgagtaaacttggtctgacagttaccaatgcttaatcagtgaggcacctatctcagcgatctgtctatttcgttcatccatagttgcctgactccccgtcgtgtagataactacgatacgggagggcttaccatctggccccagtgctgcaatgataccgcgagacccacgctcaccggctccagatttatcagcaataaaccagccagccggaagggccgagcgcagaagtggtcctgcaactttatccgcctccatccagtctattaattgttgccgggaagctagagtaagtagttcgccagttaatagtttgcgcaacgttgttgccattgctacaggcatcgtggtgtcacgctcgtcgtttggtatggcttcattcagctccggttcccaacgatcaaggcgagttacatgatcccccatgttgtgcaaaaaagcggttagctccttcggtcctccgatcgttgtcagaagtaagttggccgcagtgttatcactcatggttatggcagcactgcataattctcttactgtcatgccatccgtaagatgcttttctgtgactggtgagtactcaaccaagtcattctgagaatagtgtatgcggcgaccgagttgctcttgcccggcgtcaatacgggataataccgcgccacatagcagaactttaaaagtgctcatcattggaaaacgttcttcggggcgaaaactctcaaggatcttaccgctgttgagatccagttcgatgtaacccactcgtgcacccaactgatcttcagcatcttttactttcaccagcgtttctgggtgagcaaaaacaggaaggcaaaatgccgcaaaaaagggaataagggcgacacggaaatgttgaatactcatactcttcctttttcaatattattgaagcatttatcagggttattgtctcatgagcggatacatatttgaatgtatttagaaaaataaacaaataggggttccgcgcacatttccccgaaaagtgccacctgacgtc

SEQ ID NO: 54 - DNA, 3196 bp, synthetic construct
  misc_feature 1..3196: note = pGL4.10-CMV-MP-EPO
  source 1..3196: mol_type = other DNA
ggcctaactggccggtaccgtcgacgatatcggatccaggtctatataagcagagctcgtttagtgaaccgtcagatcgcctagatacgccatccacgctgttttgacctccatagaagatcgccaccatgggggtgcacgaatgtcctgcctggctgtggcttctcctgtccctgctgtcgctccctctgggcctcccagtcctgggcgccccaccacgcctcatctgtgacagccgagtcctggagaggtacctcttggaggccaaggaggccgagaatatcacgacgggctgtgctgaacactgcagcttgaatgagaatatcactgtcccagacaccaaagttaatttctatgcctggaagaggatggaggtcgggcagcaggccgtagaagtctggcagggcctggccctgctgtcggaagctgtcctgcggggccaggccctgttggtcaactcttcccagccgtgggagcccctgcagctgcatgtggataaagccgtcagtggccttcgcagcctcaccactctgcttcgggctctgggagcccagaaggaagccatctcccctccagatgcggcctcagctgctccactccgaacaatcactgctgacactttccgcaaactcttccgagtctactccaatttcctccggggaaagctgaagctgtacacaggggaggcctgcaggacaggggacagatgatctagagtcggggcggccggccgcttcgagcagacatgataagatacattgatgagtttggacaaaccacaactagaatgcagtgaaaaaaatgctttatttgtgaaatttgtgatgctattgctttatttgtaaccattataagctgcaataaacaagttaacaacaacaattgcattcattttatgtttcaggttcagggggaggtgtgggaggttttttaaagcaagtaaaacctctacaaatgtggtaaaatcgataaggatccgtcgaccgatgcccttgagagccttcaacccagtcagctccttccggtgggcgcggggcatgactatcgtcgccgcacttatgactgtcttctttatcatgcaactcgtaggacaggtgccggcagcgctcttccgcttcctcgctcactgactcgctgcgctcggtcgttcggctgcggcgagcggtatcagctcactcaaaggcggtaatacggttatccacagaatcaggggataacgcaggaaagaacatgtgagcaaaaggccagcaaaaggccaggaaccgtaaaaaggccgcgttgctggcgtttttccataggctccgcccccctgacgagcatcacaaaaatcgacgctcaagtcagaggtggcgaaacccgacaggactataaagataccaggcgtttccccctggaagctccctcgtgcgctctcctgttccgaccctgccgcttaccggatacctgtccgcctttctcccttcgggaagcgtggcgctttctcatagctcacgctgtaggtatctcagttcggtgtaggtcgttcgctccaagctgggctgtgtgcacgaaccccccgttcagcccgaccgctgcgccttatccggtaactatcgtcttgagtccaacccggtaagacacgacttatcgccactggcagcagccactggtaacaggattagcagagcgaggtatgtaggcggtgctacagagttcttgaagtggtggcctaactacggctacactagaagaacagtatttggtatctgcgctctgctgaagccagttaccttcggaaaaagagttggtagctcttgatccggcaaacaaaccaccgctggtagcggtggtttttttgtttgcaagcagcagattacgcgcagaaaaaaaggatctcaagaagatcctttgatcttttctacggggtctgacgctcagtggaacgaaaactcacgttaagggattttggtcatgagattatcaaaaaggatcttcacctagatccttttaaattaaaaatgaagttttaaatcaatctaaagtatatatgagtaaacttggtctgacagcggccgcaaatgctaaaccactgcagtggttaccagtgcttgatcagtgaggcaccgatctcagcgatctgcctatttcgttcgtccatagtggcctgactccccgtcgtgtagatcactacgattcgtgagggcttaccatcaggccccagcgcagcaatgatgccgcgagagccgcgttcaccggcccccgatttgtcagcaatgaaccagccagcagggagggccgagcgaagaagtggtcctgctactttgtccgcctccatccagtctatgagctgctgtcgtgatgctagagtaagaagttcgccagtgagtagtttccgaagagttgtggccattgctactggcatcgtggtatcacgctcgtcgttcggtatggcttcgttcaactctggttcccagcggtcaagccgggtcacatgatcacccatattatgaagaaatgcagtcagctccttagggcctccgatcgttgtcagaagtaagttggccgcggtgttgtcgctcatggtaatggcagcactacacaattctcttaccgtcatgccatccgtaagatgcttttccgtgaccggcgagtactcaaccaagtcgttttgtgagtagtgtatacggcgaccaagctgctcttgcccggcgtctatacgggacaacaccgcgccacatagcagtactttgaaagtgctcatcatcgggaatcgttcttcggggcggaaagactcaaggatcttgccgctattgagatccagttcgatatagcccactcttgcacccagttgatcttcagcatcttttactttcaccagcgtttcggggtgtgcaaaaacaggcaagcaaaatgccgcaaagaagggaatgagtgcgacacgaaaatgttggatgctcatactcgtcctttttcaatattattgaagcatttatcagggttactagtacgtctctcaaggataagtaagtaatattaaggtacgggaggtattggacaggccgcaataaaatatctttattttcattacatctgtgtgttggttttttgtgtgaatcgatagtactaacatacgctctccatcaaaacaaaacgaaacaaaacaaactagcaaaataggctgtccccagtgcaagtgcaggtgccagaacatttctct

SEQ ID NO: 55 - DNA, 13 bp, Mus musculus
  source 1..13: mol_type = unassigned DNA
tggcacagtgcca

SEQ ID NO: 56 - DNA, 13 bp, Homo sapiens
  source 1..13: mol_type = unassigned DNA
tgaagaggtggca

SEQ ID NO: 57 - DNA, 16 bp, Mus musculus
  source 1..16: mol_type = unassigned DNA
tcaacttgcctgacac

SEQ ID NO: 58 - DNA, 16 bp, Homo sapiens
  source 1..16: mol_type = unassigned DNA
tggactttcctgaacc

SEQ ID NO: 59 - DNA, 273 bp, synthetic construct
  misc_feature 1..273: note = Human NR1x3-Min TK
  source 1..273: mol_type = other DNA
actgtactttcctgaccctgaagagactgtactttcctgaccctgaagagactgtactttcctgaccctgaagaggatccggccccgcccagcgtcttgtcattggcgaattcgaacacgcagatgcagtcggggcggcgcggtccgaggtccacttcgcatattaaggtgacgcgtgtggcctcgaacaccgagcgaccctgcagcgacccgcttaacagcgtcaacagcgtgccgcagatctcgaggagcttggcgagattttcaggagct

SEQ ID NO: 60 - DNA, 286 bp, synthetic construct
  misc_feature 1..286: note = Human PBREM-MinTK
  source 1..286: mol_type = other DNA
actgtactttcctgaccctgaagaggtggcagcatggactttcctgaaccagatccggccccgcccagcgtcttgtcattggcgaattcgaacacgcagatgcagtcggggcggcgcggtccgaggtccacttcgcatattaaggtgacgcgtgtggcctcgaacaccgagcgaccctgcagcgacccgcttaacagcgtcaacagcgtgccgcagatctcgaggagcttggcgagattttcaggagctaaggaagctaaacatggaagatgccaaaaacattaag

SEQ ID NO: 61 - DNA, 286 bp, synthetic construct
  misc_feature 1..286: note = hNR1-mNFI-hNR2-Min TK (HMH MinTK)
  source 1..286: mol_type = other DNA
actgtactttcctgaccctggcacagtgccaccatggactttcctgaaccagatccggccccgcccagcgtcttgtcattggcgaattcgaacacgcagatgcagtcggggcggcgcggtccgaggtccacttcgcatattaaggtgacgcgtgtggcctcgaacaccgagcgaccctgcagcgacccgcttaacagcgtcaacagcgtgccgcagatctcgaggagcttggcgagattttcaggagctaaggaagctaaacatggaagatgccaaaaacattaag

SEQ ID NO: 62 - DNA, 286 bp, synthetic construct
  misc_feature 1..286: note = hNR1-mNFI mNR2-Min TK (HMM MinTK)
  source 1..286: mol_type = other DNA
actgtactttcctgaccctggcacagtgccaccatcaacttgcctgacaccgatccggccccgcccagcgtcttgtcattggcgaattcgaacacgcagatgcagtcggggcggcgcggtccgaggtccacttcgcatattaaggtgacgcgtgtggcctcgaacaccgagcgaccctgcagcgacccgcttaacagcgtcaacagcgtgccgcagatctcgaggagcttggcgagattttcaggagctaaggaagctaaacatggaagatgccaaaaacattaag

SEQ ID NO: 63 - DNA, 286 bp, synthetic construct
  misc_feature 1..286: note = mNR1-hNFI-mNR2-Min TK (MHM MinTK)
  source 1..286: mol_type = other DNA
tctgtactttcctgaccttgaagaggtggcaccatcaacttgcctgacaccgatccggccccgcccagcgtcttgtcattggcgaattcgaacacgcagatgcagtcggggcggcgcggtccgaggtccacttcgcatattaaggtgacgcgtgtggcctcgaacaccgagcgaccctgcagcgacccgcttaacagcgtcaacagcgtgccgcagatctcgaggagcttggcgagattttcaggagctaaggaagctaaacatggaagatgccaaaaacattaag

SEQ ID NO: 64 - DNA, 286 bp, synthetic construct
  misc_feature 1..286: note = mNR1-hNFI hNR2-Min TK (MHH MinTK)
  source 1..286: mol_type = other DNA
tctgtactttcctgaccttgaagaggtggcagcatggactttcctgaaccagatccggccccgcccagcgtcttgtcattggcgaattcgaacacgcagatgcagtcggggcggcgcggtccgaggtccacttcgcatattaaggtgacgcgtgtggcctcgaacaccgagcgaccctgcagcgacccgcttaacagcgtcaacagcgtgccgcagatctcgaggagcttggcgagattttcaggagctaaggaagctaaacatggaagatgccaaaaacattaag

SEQ ID NO: 65 - DNA, 330 bp, synthetic construct
  misc_feature 1..330: note = hPB-SV40
  source 1..330: mol_type = other DNA
actgtactttcctgaccctgaagaggtggcagcatggactttcctgaaccagctgggagttcgtagacggactagcccgggctcgagatctgcgatctgcatctcaattagtcagcaaccatagtcccgcccctaactccgcccatcccgcccctaactccgcccagttccgcccattctccgccccatcgctgactaattttttttatttatgcagaggccgaggccgcctcggcctctgagctattccagaagtagtgaggaggcttttttggaggcctaggcttttgcaaaaagcttggcattccggtactgttggtaaagccaccc

SEQ ID NO: 66 - DNA, 330 bp, synthetic construct
  misc_feature 1..330: note = MHM-SV40
  source 1..330: mol_type = other DNA
tctgtactttcctgaccttgaagaggtggcaccatcaacttgcctgacaccgctgggagttcgtagacggactagcccgggctcgagatctgcgatctgcatctcaattagtcagcaaccatagtcccgcccctaactccgcccatcccgcccctaactccgcccagttccgcccattctccgccccatcgctgactaattttttttatttatgcagaggccgaggccgcctcggcctctgagctattccagaagtagtgaggaggcttttttggaggcctaggcttttgcaaaaagcttggcattccggtactgttggtaaagccaccc

SEQ ID NO: 67 - DNA, 401 bp, synthetic construct
  misc_feature 1..401: note = 2xhPB SV40
  source 1..401: mol_type = other DNA
actgtactttcctgaccctgaagaggtggcagcatggactttcctgaaccacattactcgcatccattctcactgtactttcctgaccctgaagaggtggcagcatggactttcctgaaccagctgggagttcgtagacggactagcccgggctcgagatctgcgatctgcatctcaattagtcagcaaccatagtcccgcccctaactccgcccatcccgcccctaactccgcccagttccgcccattctccgccccatcgctgactaattttttttatttatgcagaggccgaggccgcctcggcctctgagctattccagaagtagtgaggaggcttttttggaggcctaggcttttgcaaaaagcttggcattccggtactgttggtaaagccaccc

SEQ ID NO: 68 - DNA, 353 bp, synthetic construct
  misc_feature 1..353: note = 2xMHM-MinTK
  source 1..353: mol_type = other DNA
tctgtactttcctgaccttgaagaggtggcaccatcaacttgcctgacacccattactcgcatccattctctctgtactttcctgaccttgaagaggtggcaccatcaacttgcctgacaccgctgggagttcgtagacggagatccggccccgcccagcgtcttgtcattggcgaattcgaacacgcagatgcagtcggggcggcgcggtccgaggtccacttcgcatattaaggtgacgcgtgtggcctcgaacaccgagcgaccctgcagcgacccgcttaacagcgtcaacagcgtgccgcagatctcgaggagcttggcgagattttcaggagctaaggaagctaaac

SEQ ID NO: 69 - DNA, 401 bp, synthetic construct
  misc_feature 1..401: note = 2xMHM-SV40
  source 1..401: mol_type = other DNA
tctgtactttcctgaccttgaagaggtggcaccatcaacttgcctgacacccattactcgcatccattctctctgtactttcctgaccttgaagaggtggcaccatcaacttgcctgacaccgctgggagttcgtagacggactagcccgggctcgagatctgcgatctgcatctcaattagtcagcaaccatagtcccgcccctaactccgcccatcccgcccctaactccgcccagttccgcccattctccgccccatcgctgactaattttttttatttatgcagaggccgaggccgcctcggcctctgagctattccagaagtagtgaggaggcttttttggaggcctaggcttttgcaaaaagcttggcattccggtactgttggtaaagccaccc

SEQ ID NO: 70 - DNA, 424 bp, synthetic construct
  misc_feature 1..424: note = 3xhPB-minTK
  source 1..424: mol_type = other DNA
actgtactttcctgaccctgaagaggtggcagcatggactttcctgaaccacattactcgcatccattctcactgtactttcctgaccctgaagaggtggcagcatggactttcctgaaccagcactgaaggtcctcaatcgactgtactttcctgaccctgaagaggtggcagcatggactttcctgaaccagctgggagttcgtagacggagatccggccccgcccagcgtcttgtcattggcgaattcgaacacgcagatgcagtcggggcggcgcggtccgaggtccacttcgcatattaaggtgacgcgtgtggcctcgaacaccgagcgaccctgcagcgacccgcttaacagcgtcaacagcgtgccgcagatctcgaggagcttggcgagattttcaggagctaaggaagctaaac

SEQ ID NO: 71 - DNA, 472 bp, synthetic construct
  misc_feature 1..472: note = 3xhPB-SV40
  source 1..472: mol_type = other DNA
actgtactttcctgaccctgaagaggtggcagcatggactttcctgaaccacattactcgcatccattctcactgtactttcctgaccctgaagaggtggcagcatggactttcctgaaccagcactgaaggtcctcaatcgactgtactttcctgaccctgaagaggtggcagcatggactttcctgaaccagctgggagttcgtagacggactagcccgggctcgagatctgcgatctgcatctcaattagtcagcaaccatagtcccgcccctaactccgcccatcccgcccctaactccgcccagttccgcccattctccgccccatcgctgactaattttttttatttatgcagaggccgaggccgcctcggcctctgagctattccagaagtagtgaggaggcttttttggaggcctaggcttttgcaaaaagcttggcattccggtactgttggtaaagccaccc

SEQ ID NO: 72 - DNA, 51 bp, synthetic construct
  misc_feature 1..51: note = HMH hybrid
  source 1..51: mol_type = other DNA
actgtactttcctgaccctggcacagtgccaccatggactttcctgaacca

SEQ ID NO: 73 - DNA, 51 bp, synthetic construct
  misc_feature 1..51: note = HMM hybrid
  source 1..51: mol_type = other DNA
actgtactttcctgaccctggcacagtgccaccatcaacttgcctgacacc

SEQ ID NO: 74 - DNA, 51 bp, synthetic construct
  misc_feature 1..51: note = MHM hybrid
  source 1..51: mol_type = other DNA
tctgtactttcctgaccttgaagaggtggcaccatcaacttgcctgacacc

SEQ ID NO: 75 - DNA, 51 bp, synthetic construct
  misc_feature 1..51: note = MHH hybrid
  source 1..51: mol_type = other DNA
tctgtactttcctgaccttgaagaggtggcagcatggactttcctgaacca

SEQ ID NO: 76 - DNA, 101 bp, synthetic construct
  misc_feature 1..101: note = 2x mouse PBREM CREs
  misc_feature 51..52: note = optional spacer
  source 1..101: mol_type = other DNA
tctgtactttcctgaccttggcacagtgccaccatcaacttgcctgacaccctgtactttcctgaccttggcacagtgccaccatcaacttgcctgacacc

SEQ ID NO: 77 - DNA, 204 bp, synthetic construct
  misc_feature 1..204: note = 3x mouse PBREM CREs
  misc_feature 51..52: note = optional spacer
  misc_feature 102..103: note = optional spacer
  misc_feature 153..154: note = optional spacer
  source 1..204: mol_type = other DNA
tctgtactttcctgaccttggcacagtgccaccatcaacttgcctgacacctctgtactttcctgaccttggcacagtgccaccatcaacttgcctgacacctctgtactttcctgaccttggcacagtgccaccatcaacttgcctgacacctctgtactttcctgaccttggcacagtgccaccatcaacttgcctgacacc

SEQ ID NO: 78 - DNA, 101 bp, synthetic construct
  misc_feature 1..101: note = 2x MHM hybrids CREs
  misc_feature 50..51: note = optional spacer
  source 1..101: mol_type = other DNA
ctgtactttcctgaccttgaagaggtggcaccatcaacttgcctgacacctctgtactttcctgaccttgaagaggtggcaccatcaacttgcctgacacc

SEQ ID NO: 79 - DNA, 102 bp, synthetic construct; identical to SEQ ID NO: 47
  misc_feature 1..102: note = 2x human PBREM CREs
  misc_feature 51..52: note = optional spacer
  source 1..102: mol_type = other DNA

SEQ ID NO: 80 - DNA, 153 bp, synthetic construct; identical to SEQ ID NO: 46
  misc_feature 1..153: note = 3x human PBREM CREs
  misc_feature 51..52: note = optional spacer
  misc_feature 102..103: note = optional spacer
  source 1..153: mol_type = other DNA

SEQ ID NO: 81 - DNA, 122 bp, synthetic construct
  misc_feature 1..122: note = 2x mouse PBREM CREs
  source 1..122: mol_type = other DNA
tctgtactttcctgaccttggcacagtgccaccatcaacttgcctgacacccattactcgcatccattctctctgtactttcctgaccttggcacagtgccaccatcaacttgcctgacacc

SEQ ID NO: 82 - DNA, 264 bp, synthetic construct
  misc_feature 1..264: note = 3x mouse PBREM
  source 1..264: mol_type = other DNA
tctgtactttcctgaccttggcacagtgccaccatcaacttgcctgacacccattactcgcatccattctctctgtactttcctgaccttggcacagtgccaccatcaacttgcctgacaccgcactgaaggtcctcaatcgtctgtactttcctgaccttggcacagtgccaccatcaacttgcctgacaccctgacctcctgccagcaatatctgtactttcctgaccttggcacagtgccaccatcaacttgcctgacacc

SEQ ID NO: 83 - DNA, 121 bp, synthetic construct
  misc_feature 1..121: note = 2x MHM hybrids
  source 1..121: mol_type = other DNA
ctgtactttcctgaccttgaagaggtggcaccatcaacttgcctgacacccattactcgcatccattctctctgtactttcctgaccttgaagaggtggcaccatcaacttgcctgacacc

SEQ ID NO: 84 - DNA, 122 bp, synthetic construct
  misc_feature 1..122: note = 2x human PBREM
  source 1..122: mol_type = other DNA
actgtactttcctgaccctgaagaggtggcagcatggactttcctgaaccacattactcgcatccattctcactgtactttcctgaccctgaagaggtggcagcatggactttcctgaacca

SEQ ID NO: 85 - DNA, 193 bp, synthetic construct
  misc_feature 1..193: note = 3x human PBREM
  source 1..193: mol_type = other DNA
actgtactttcctgaccctgaagaggtggcagcatggactttcctgaaccacattactcgcatccattctcactgtactttcctgaccctgaagaggtggcagcatggactttcctgaaccagcactgaaggtcctcaatcgactgtactttcctgaccctgaagaggtggcagcatggactttcctgaacca

SEQ ID NO: 86 - DNA, 18 bp, Mus musculus
  source 1..18: mol_type = unassigned DNA
tctgtactttcctgacct

SEQ ID NO: 87 - DNA, 18 bp, Homo sapiens
  source 1..18: mol_type = unassigned DNA
actgtactttcctgaccc

SEQ ID NO: 88 - DNA, 16 bp, Mus musculus
  source 1..16: mol_type = unassigned DNA
tggcacagtgccacca

SEQ ID NO: 89 - DNA, 16 bp, Homo sapiens
  source 1..16: mol_type = unassigned DNA
tgaagaggtggcagca

SEQ ID NO: 90 - DNA, 17 bp, Mus musculus
  source 1..17: mol_type = unassigned DNA
tcaacttgcctgacacc

SEQ ID NO: 91 - DNA, 17 bp, Homo sapiens
  source 1..17: mol_type = unassigned DNA
tggactttcctgaacca